European Patent Application EP 4 223 773 A2, published August 9, 2023. Title: Methods. Applicant: Institut Pasteur. The sequence listing filed with the application follows.

SEQUENCE LISTING (156 sequences)

SEQ ID NO: 1 - protein, 120 aa, synthetic construct
  REGION 1..120: note = Full sequence of antibody C8 heavy chain
EVQLVESGGGLVQPGGSLRLSCSASGFTFSTYSMHWVRQAPGKGLEYVSAITGEGDSAFYADSVKGRFTISRDNSKNTLYFEMNSLRPEDTAVYYCVGGYSNFYYYYTMDVWGQGTTVTV

SEQ ID NO: 2 - protein, 126 aa, synthetic construct
  REGION 1..126: note = Full sequence of antibody C10 heavy chain
EVQLVESGAEVKKPGASVKVSCKASGYTFTSYAMHWVRQAPGQRLEWMGWINAGNGNTKYSQKFQDRVTITRDTSASTAYMELSSLRSEDTAIYYCARDKVDDYGDYWFPTLWYFDYWGQGTLVTV

SEQ ID NO: 3 - protein, 131 aa, synthetic construct
  REGION 1..131: note = Full sequence of antibody A11 heavy chain
EVQLVESGGGLVRPGGSLRLSCAASGFSYSNHWMHWVRQAPGKGLVWVSRINSDGSTRNYADFVKGRFTISRDNAENTLYLEMNSLTADDTAVYYCVRDGVRFYYDSTGYYPDSFFKYGMDVWGQGTTVTV

SEQ ID NO: 4 - protein, 128 aa, synthetic construct
  REGION 1..128: note = Full sequence of antibody B7 heavy chain
EVQLVESGGGLVQPGGSLKLSCAASGFTFSSHWMHWVRQAPGKGLVWVSRTNSDGSSTSYADSVKGRFMISRDNSKNTVYLHMNGLRAEDTAVYFCARDGVRYYYDSTGYYPDNFFQYGLDVWGQGTT

SEQ ID NO: 5 - protein, 5 aa, synthetic construct
  REGION 1..5: note = C8 CDR H1
TYSMH

SEQ ID NO: 6 - protein, 17 aa, synthetic construct
  REGION 1..17: note = C8 CDR H2
AITGEGDSAFYADSVKG

SEQ ID NO: 7 - protein, 8 aa, synthetic construct
  REGION 1..8: note = C8 CDR H3
GYSNFYYY

SEQ ID NO: 8 - protein, 5 aa, synthetic construct
  REGION 1..5: note = C10 CDR H1
SYAMH

SEQ ID NO: 9 - protein, 17 aa, synthetic construct
  REGION 1..17: note = C10 CDR H2
WINAGNGNTKYSQKFQD

SEQ ID NO: 10 - protein, 15 aa, synthetic construct
  REGION 1..15: note = C10 CDR H3
DKVDDYGDYWFPTLW

SEQ ID NO: 11 - protein, 5 aa, synthetic construct
  REGION 1..5: note = A11 CDR H1
NHWMH

SEQ ID NO: 12 - protein, 17 aa, synthetic construct
  REGION 1..17: note = A11 CDR H2
RINSDGSTRNYADFVKG

SEQ ID NO: 13 - protein, 20 aa, synthetic construct
  REGION 1..20: note = A11 CDR H3
DGVRFYYDSTGYYPDSFFKY

SEQ ID NO: 14 - protein, 5 aa, synthetic construct
  REGION 1..5: note = B7 CDR H1
SHWMH

SEQ ID NO: 15 - protein, 17 aa, synthetic construct
  REGION 1..17: note = B7 CDR H2
RTNSDGSSTSYADSVKG

SEQ ID NO: 16 - protein, 20 aa, synthetic construct
  REGION 1..20: note = B7 CDR H3
DGVRYYYDSTGYYPDNFFQY

SEQ ID NO: 17 - protein, 11 aa, synthetic construct
  REGION 1..11: note = C8-CDR L1
RASQSISTFLA

SEQ ID NO: 18 - protein, 7 aa, synthetic construct
  REGION 1..7: note = C8 CDR L2
DASTRAT

SEQ ID NO: 19 - protein, 10 aa, synthetic construct
  REGION 1..10: note = C8 CDR L3
QQRYNWPPYT

SEQ ID NO: 20 - protein, 14 aa, synthetic construct
  REGION 1..14: note = C10 CDR L1
TGTSSDVGGFNYVS

SEQ ID NO: 21 - protein, 7 aa, synthetic construct
  REGION 1..7: note = C10 CDR L2
DVTSRPS

SEQ ID NO: 22 - protein, 11 aa, synthetic construct
SSHTSRGTWVF

SEQ ID NO: 23 - protein, 14 aa, synthetic construct
  REGION 1..14: note = A11 CDR L1
TGTSSNADTYNLVS

SEQ ID NO: 24 - protein, 7 aa, synthetic construct
  REGION 1..7: note = A11 CDR L2
EGTKRPS

SEQ ID NO: 25 - protein, 11 aa, synthetic construct
  REGION 1..11: note = A11 CDR L3
CSYATSRTLVF

SEQ ID NO: 26 - protein, 14 aa, synthetic construct
  REGION 1..14: note = B7 CDR L1
TGISSDVETYNLVS

SEQ ID NO: 27 - protein, 7 aa, synthetic construct
  REGION 1..7: note = B7 CDR L2
EASKRPS

SEQ ID NO: 28 - protein, 10 aa, synthetic construct
  REGION 1..10: note = B7 CDR L3
CSYAGGKSLV

SEQ ID NO: 29 - protein, 495 aa, synthetic construct
  REGION 1..495: note = Full length envelope protein sequence DENV1
MRCVGIGNRDFVEGLSGGTWVDVVLEHGSCVTTMAKDKPTLDIELLKTEVTNPAVLRKLCIEAKISNTTTDSRCPTQGEATLVEEQDANFVCRRTFVDRGWGNGCGLFGKGSLITCAKFKCVTKLEGKIVQYENLKYSVIVTVHTGDQHQVGNETTEHGTIATITPQAPTSEIQLTDYGALTLDCSPRTGLDFNEMVLLTMKEKSWLVHKQWFLDLPLPWTSGASTPQETWNREDLLVTFKTAHAKKQEVVVLGSQEGAMHTALTGATEIQTSGTTKIFAGHLKCRLKMDKLTLKGMSYVMCTGSFKLEKEVAETQHGTVLVQVKYEGTDAPCKIPFSTQDEKGVTQNGRLITANPIVTDKEKPVNIEAEPPFGESYIVVGAGEKALKLSWFKKGSSIGKMLEATARGARRMAILGDTAWDFGSIGGVFTSVGKLVHQIFGTAYGVLFSGVSWTMKIGIGILLTWLGLNSRSTSLSMTCIAVGMVTLYLGVMVQA

SEQ ID NO: 30 - skipped

SEQ ID NO: 31 - protein, 495 aa, synthetic construct
  REGION 1..495: note = Full length envelope protein sequence DENV2
MRCIGMSNRDFVEGVSGGSWVDIVLEHGSCVTTMAKNKPTLDFELIKTEAKQPATLRKYCIEAKLTNTTTESRCPTQGEPSLNEEQDKRFVCKHSMVDRGWGNGCGLFGKGGIVTCAMFRCKKNMEGKVVQPENLEYTIVITPHSGEEHAVGNDTGKHGKEIKITPQSSITEAELTGYGTVTMECSPRTGLDFNEMVLLQMENKAWLVHRQWFLDLPLPWLPGADTQGSNWIQKETLVTFKNPHAKKQDVVVLGSQEGAMHTALTGATEIQMSSGNLLFTGHLKCRLRMDKLQLKGMSYSMCTGKFKVVKEIAETQHGTIVIRVQYEGDGSPCKIPFEIMDLEKRHVLGRLITVNPIVTEKDSPVNIEAEPPFGDSYIIIGVEPGQLKLNWFKKGSSIGQMFETTMRGAKRMAILGDTAWDFGSLGGVFTSIGKALHQVFGAIYGAAFSGVSWTMKILIGVIITWIGMNSRSTSLSVTLVLVGIVTLYLGVMVQA

SEQ ID NO: 32 - skipped

SEQ ID NO: 33 - protein, 493 aa, synthetic construct
  REGION 1..493: note = Full length envelope protein sequence DENV3
MRCVGVGNRDFVEGLSGATWVDVVLEHGGCVTTMAKNKPTLDIELQKTEATQLATLRKLCIEGKITNITTDSRCPTQGEAILPEEQDQNYVCKHTYVDRGWGNGCGLFGKGSLVTCAKFQCLESIEGKVVQHENLKYTVIITVHTGDQHQVGNETQGVTAEITSQASTAEAILPGYGTLGLECSPRTGLDFNEMILLTMKNKAWMVHRQWFFDLPLPWTSGATTETPTWNRRELLVTFKNAHAKKQEVVVLGSQEGAMHTALTGATEIQTSGGTSIFAGHLKCRLKMDKLELKGMSYAMCLNTFVLKKEVSETQHGTILIKVEYKGEDAPCKIPFSTEDGQGKAHNGRLITANPVVTKKEEPVNIEAEPPFGESNIVIGIGDKALKINWYRKGSSIGKMFEATARGARRMAILGDTAWDFGSVGGVLNSLGKMVHQIFGSAYTALFSGVSWIMKIGIGVLLTWIGLNSKNTSMSFSCIAIGIITLYLGVVVQA

SEQ ID NO: 34 - skipped

SEQ ID NO: 35 - protein, 495 aa, synthetic construct
  REGION 1..495: note = Full length envelope protein sequence DENV4
MRCVGVGNRDFVEGVSGGAWVDLVLEHGGCVTTMAQGKPTLDFELIKTTAKEVALLRTYCIEASISNITTATRCPTQGEPYLKEEQDQQYICRRDVVDRGWGNGCGLFGKGGVVTCAKFSCSGKITGNLVQIENLEYTVVVTVHNGDTHAVGNDIPNHGVTATITPRSPSVEVKLPDYGELTLDCEPRSGIDFNEMILMKMKKKTWLVHKQWFLDLPLPWAAGADTSEVHWNYKERMVTFKVPHAKRQDVIVLGSQEGAMHSALTGATEVDSGDGNHMFAGHLKCKVRMEKLRIKGMSYTMCSGKFSIDKEMAETQHGTTVVKVKYEGAGAPCKVPIEIRDVNKEKVVGRIISSTPFAEYTNSVTNIELEPPFGDSYIVIGVGDSALTLHWFRKGSSIGKMLESTYRGVKRMAILGETAWDFGSVGGLFTSLGKAVHQVFGSVYTTMFGGVSWMVRILIGFLVLWIGTNSRNTSMAMTCIAVGGITLFLGFTVHA

SEQ ID NO: 36 - skipped

SEQ ID NO: 37 - protein, 108 aa, synthetic construct
  REGION 1..108: note = C8 light chain
EIVLTQSPATLSLSPGERATLSCRASQSISTFLAWYQHKPGQAPRLLIYDASTRATGVPARFSGSRSGTDFTLTISTLEPEDFAVYYCQQRYNWPPYTFGQGTKVEIK

SEQ ID NO: 38 - protein, 110 aa, synthetic construct
  REGION 1..110: note = C10 light chain
QSALTQPASVSGSPGQSITISCTGTSSDVGGFNYVSWFQQHPGKAPKLMLYDVTSRPSGVSSRFSGSKSGNTASLTISGLQAEDEADYYCSSHTSRGTWVFGGGTKLTVL

SEQ ID NO: 39 - protein, 110 aa, synthetic construct
  REGION 1..110: note = A11 light chain
QSVLTQPASVSGSPGQSITISCTGTSSNADTYNLVSWYQQRPGKAPKLMIYEGTKRPSGVSNRFSASKSATAASLTISGLQPEDEADYYCCSYATSRTLVFGGGTKLTVV

SEQ ID NO: 40 - protein, 110 aa, synthetic construct
  REGION 1..110: note = B7 light chain
QSALTQPASVSGSPGQSITISCTGISSDVETYNLVSWYEQHPGKAPKLIIYEASKRPSGVSNRFSGSKSGNTASLAISGLQAEDEADYYCCSYAGGKSLVFGGGTRLTVL

SEQ ID NO: 41 - protein, 128 aa, synthetic construct
  REGION 1..128: note = A12 heavy chain
EVQLVESGSELKKPGASVKVSCRASGFTFTSYTFNWVRQAPGQGLEWMGWIDTKSGRPTYAQGFTGRFVLSLDTSVSTAYLQINSLKVEDTAMYYCARVHTGGYPPELRYYYYGMDVWGQGTTVTVSS

SEQ ID NO: 42 - protein, 122 aa, synthetic construct
  REGION 1..122: note = B10 heavy chain
EVQLVESGGGLVQPGGSLRLSCSASGFTFSTYSMHWVRQAPGKGLEYVSAITTDGNSAFYADSVKGRFTISRDNSKNTMYFHMNSLRPEDTAVYYCVGGYSSFYYYYTMDVWGQGTTVTVSS

SEQ ID NO: 43 - protein, 122 aa, synthetic construct
  REGION 1..122: note = B11 heavy chain
QVQLVESGGGLVQPGGSLRLSCSASGFTFSTYSMHWVRQAPGKGLEYVSAITTDGDSAFYADSVKGRFTISRDNSKNTMFFHMSNLRPEDTAVYYCVGGYSSFYYYYTLDVWGQGTTVTVSS

SEQ ID NO: 44 - protein, 122 aa, synthetic construct
  REGION 1..122: note = C9 heavy chain
EVQLVESEGGLVQPGGSLRLSCSASGFTFSTYSMHWVRQAPGKGLEYVSAITTNGDSTFYADSVKGRFTISRDNSKNTLYFQMSSLRAEDTGVYYCVGGYSSFYYYYTMDVWGQGTTVTVSS

SEQ ID NO: 45 - protein, 124 aa, synthetic construct
  REGION 1..124: note = A2 heavy chain
EVQLVQSGPEMRKPGASVKVSCKASGYTFTSHGINWVRQVPGQGPEWMGWSSSYTDNTNYAQKFKGRVTMTTDPSTSTAYMELRSLRSDDTAIYFCARGFYSGSYYPTAPFDIWGQGTLVTVSS

SEQ ID NO: 46 - protein, 124 aa, synthetic construct
  REGION 1..124: note = A5 heavy chain
EVQLVQSGAEVKKPGASVKVSCKASGYTFTTYGLSWVRQAPGQGLEWMGWCSSYNDNTNYAQKFKGRVTMTTDTSTNTAYMELRSLRSDDTAVYYCARVFYSGSYYPNSPFDYWGQGTLVTVSS

SEQ ID NO: 47 - protein, 124 aa, synthetic construct
  REGION 1..124: note = A7 heavy chain
QVQLQESGPGLVKPSQTLSLTCTVSGDSISSNNYQWNWIRQPAGKGLEWLGRIDTTGSTNYNPSLKSRISISIDTSKKQFSLRLNSVTAADTAVYYCARSLWSGELWGGPLGYWGQGTLVTVSS

SEQ ID NO: 48 - protein, 125 aa, synthetic construct
  REGION 1..125: note = A8 heavy chain
EVQLVESGAEVKNPGASVKVSCKASGYTFIGYYIHWVRQAPGQGLEWMGWINPNSGATYSAQKFQGRVTLTGDASPSTVYMELSSLRSDDTAIYYCAGRSYNWNDVFYYYYMDVWGQGTTVTVSS

SEQ ID NO: 49 - protein, 125 aa, synthetic construct
  REGION 1..125: note = B10 heavy chain
EVQLVESGPGLVKPSETLSLTCTISGVSISDYYWTWIRQPPGKGLEWIGNIYNTGSTNYNPSLKSRVAIWMDTSKNKFSLRLTSVTSADTAVYYCARVEGGPKYYFGSGDFYNLWGRGSLVTVSS

SEQ ID NO: 50 - protein, 125 aa, synthetic construct
  REGION 1..125: note = C2 heavy chain
SQVQLVQSGAELKKPGASVKVSCKTSGYTFSYYIHWVRQAPGQGLEWMAMINPTSGSTSYAQRFQGRVTMTRDTPTNTVYMEVRSLRSDDTAVYFCASRGYNWNDVQYYYTMDVWGQGTTVTVSS

SEQ ID NO: 51 - protein, 125 aa, synthetic construct
  REGION 1..125: note = D4 heavy chain
SEVQLVQSGAELKKPGASVKVSCKASGYTFSYYIHWVRQAPGQGLEWMAIINPTSGSTSYAQRFQGRVTMTRDTSTNTVYMELSSLISEDTAVYYCASRGYNWNDVHYYYTMDVWGQGTTVTVSS

SEQ ID NO: 52 - protein, 114 aa, synthetic construct
  REGION 1..114: note = B11 heavy chain
QVQLVESGAEVKKPGSSVKVSCKASGYTFTTYGLSWVRQAPGQGLEWMGWCSSYEDNTNYAPRFKGRVTMTTDTSTNTAYMELRSLRFDDTAVYYCARVFYSGSYYPNSPFDSW

SEQ ID NO: 53 - protein, 122 aa, synthetic construct
  REGION 1..122: note = A2 heavy chain
QVQLVESGGGLVQPGGSLRLSCSASGFTFSTYSMHWVRQAPGKGLEYISAITTDGDSAFYADSVKGRFTISRDNSKNTMYFHMNSLRPEDTAVYYCVGGYSSFYYYYTMDVWGQGTTVTVSS

SEQ ID NO: 54 - protein, 124 aa, synthetic construct
  REGION 1..124: note = A4 heavy chain
EVQLVESGAEVKKPGASVKVSCKASGYTFTSYGINWVRQAPGQGLEWMGWISSDSGHTNYARKLKGRVTMTTDTSTTTAYMELRSLRSDDTAVYYCARGLYSVSYYPTSPFDYWGQGSTVTVSS

SEQ ID NO: 55 - protein, 124 aa, synthetic construct
  REGION 1..124: note = A5 heavy chain
QVQLVESGAEVKKPGSSVKVSCRASGYTFTTYGLSWVRQAPGQGLEWMGWCSSYNDNTNYAQKFKGRVTMTTDTSTNTAYMELRSLRSDDTAVYYCARVFYSGSYYPNSPFDSWGQGTLVTVSS

SEQ ID NO: 56 - protein, 122 aa, synthetic construct
  REGION 1..122: note = A9 heavy chain
EVQLVESGGGLVQPGGSLRLSCSASGFTFSTYSMHWVRQAPGKGLEYVSAITTDGDSAFYADSVKGRFTISRDNSKNTMYFHMNSVRPEDTAVYYCVGGYSSFYYYYTMDVWGQGTTVTVSS

SEQ ID NO: 57 - protein, 122 aa, synthetic construct
  REGION 1..122: note = B2 heavy chain
EVQLVESGGGLVQPGGSLRLSCSASGFTFSTYSMHWVRQAPGKGLEYVSAITTDGDSAFYADSVKGRFTISRDNSKNTMYFHMNSLRPEDTAVYYCVGGYSSFYYYYTMDVWGQGTTVTVSS

SEQ ID NO: 58 - protein, 122 aa, synthetic construct
  REGION 1..122: note = B3 heavy chain
EVQLLESGGGLVQPGGSLRLSCSASGFTFSTYSMHWVRQAPGKGLEYVSAISTDGDSAFYADSVKGRFTISRDNSKNTLYFHMSSLRAEDTAVYYCLGGYSTFYYYYTMDVWGQGTTVTVSS

SEQ ID NO: 59 - protein, 112 aa, synthetic construct
  REGION 1..112: note = B4 heavy chain
QVQLVESGGGLVQPGGSLRLSCSASGFPFSTYSMHWVRQAPGKGLEYVSAITTNGDSTFYADSVKGRFTISRDNSKNTVYFQLSSLRAEDTAVYYCVGGYSSFYFYYTMDVW

SEQ ID NO: 60 - protein, 124 aa, synthetic construct
  REGION 1..124: note = B7 heavy chain
EVQLVQSGAEVKKPGASVKVSCKASGYTYTNYGLSWVRQAPGQGLEWMGWMSSYNDNTNYSQKFKGRVTMTTDPSTTTAYMELRSLRSDDTAVYYCARGLYSGSHYPTSPLDYWGQGTLVTVSS

SEQ ID NO: 61 - protein, 122 aa, synthetic construct
  REGION 1..122: note = B11 heavy chain
EVQLVESGGGLVQPGGSLRLSCSASGFTFTTYSLHWVRQTPGKGLEYVSAITTDGDSAFYADSVKGRFTISRDNSKNTMYFHMSSLRPEDTAVYYCVGGYSSFYYFYTVDVWGQGTTVTVSF

SEQ ID NO: 62 - protein, 125 aa, synthetic construct
  REGION 1..125: note = C4 heavy chain
SQVQLVESGAELKKPGASVKVSCKASGYTFSYYMHWVRQAPGQGLEWMAIINPTSGSTTYAQRFQGRVTMTRDTSTSTVYMELSSLRSEDTAVYYCASRGYNWNDVHYYYTMDVWGQGTTVTVSS

SEQ ID NO: 63 - protein, 131 aa, synthetic construct
  REGION 1..131: note = B10 heavy chain
EVQLVESGPEVKKPGASVKVSCKTSGYTFINYYIHWVRQAPGQGLEWLGLINPRGGNTNYAEKFEDRVTMTRDTSTSTVNMELSSLTSEDTAVYYCARPLAHTYDFWSGYHRATGYGMDVWGQGTTVTVSS

SEQ ID NO: 64 - protein, 126 aa, synthetic construct
  REGION 1..126: note = P6A1 heavy chain
EVQLVESGGGLVQPGGSLRLSCAAFGFTFVNYAMNWVRQAPGKGPEWVAVIYAAGDGANYGDSVKGRFTISRDNSRNTLYLQMNSLRAEDTAIYYCAKPAHYDDSGYPYMAYFDSWGQGTLVTVSS

SEQ ID NO: 65 - protein, 126 aa, synthetic construct
  REGION 1..126: note = P6A3 heavy chain
QVQLVQSGAEVKKPGSSVKVSCKASGGFFSSYAITWVRQAPGQGLEWMGGIIPDYDSAKYAQKFQGRVTITADESTSTAYLELRSLRSEDTAVYYCARRHCSSTSCSDPWTFFPSWGQGTLVTSPQ

SEQ ID NO: 66 - protein, 126 aa, synthetic construct
  REGION 1..126: note = P6A12 heavy chain
EVQLVESGAEMKKPGSSVKVSCKASGATFTSFAMYWVRQAPGQGLEWMGRIIPMFASAEYAQKFQGRLTMTADESTTTAYMELSSLRSDDTAVYYCAGRYCSSTSCSDPWTYFPHWGQGTLVTVSS

SEQ ID NO: 67 - protein, 130 aa, synthetic construct
  REGION 1..130: note = P6B4 heavy chain
EVQLVQSGATVRKPGASVTISCKTSGYTFTDYALHWVRQAPGQRLEWMGWLIPGSGYTKFAENFQGRVTITRATSAHTAYMELSNLRSEDTAVYYCARWGGDCNAGSCYGPYQYRGLDAWGQGTTVTVSS

SEQ ID NO: 68 - protein, 125 aa, synthetic construct
  REGION 1..125: note = P6B5 heavy chain
EVQLVQSGAEVKKPGASVKVSCKASGYSFIGYYLHWVRQAPGQGLEWMGRINPNSGGIDYGQTFQGRVTMTRDMSSSTVYLELTRLRSDDTARYYCAGRSDNWNDVYYNYALDVWGQGTTVTVSS

SEQ ID NO: 69 - protein, 129 aa, synthetic construct
  REGION 1..129: note = P6B11 heavy chain
EVQLLESGGGVVQPGRSLKLSCAASGFTFSGYAMHWVRQAPGKGLEWLAVISYDATTTYYTPSVKGRFTISRDNSKNTLYLQINSLRAEDAAVYYCAKEISYCGGDCQNFFFYYNMDVWGQGTTVTVSS

SEQ ID NO: 70 - protein, 128 aa, synthetic construct
  REGION 1..128: note = P6C4 heavy chain
QVQLVQSGAEVKKPGASVKVSCKASGYTFTAYYIHWVRQAPGQGLEWMGSINPNNGGTNYAQGFQGRVTMTRDTSIRTVYMELSKLRSDDTALYYCARDLGAMGYYLCSAGNCPFDYWGQGTLVTVSS

SEQ ID NO: 71 - protein, 133 aa, synthetic construct
  REGION 1..133: note = B8 heavy chain
QVQLVESGGALVKPGGSLRLSCAASGFTFRSHWMHWVRQAPGKGLVWVSRINSDGSSTNYADFVKGRFTTSRDNAENTLYLEMNSLTADDTAVYYCVRDGVRYYYDSSGYYPDSFFKYGMDVWGQGTTVTVSS

SEQ ID NO: 72 - protein, 126 aa, synthetic construct
  REGION 1..126: note = C2 heavy chain
EVQLVESGGGLVQPGGSLRLSCAASGFTFRSSAMYWVRQAPGKGLEFVSCIRSNGVTHYADSVKGRFTISRDNSKNTLHLQMGGLRPDDMAVYYCTRDDGPYSGYDWPWASSMDVWGQGTTVTVSS

SEQ ID NO: 73 - protein, 133 aa, synthetic construct
  REGION 1..133: note = D8 heavy chain
EVQLVESGGGLVQPGGSLRLSCAASGFIFSNHWMHWVRQAPGKGLVWVSRTNSDGSSTSYADFVKGRFTISRDNAKNTLHLQINSLRADDTAVYYCARDGVRYYYDSTGYYPDSYYEYGLDVWGQGTTVTVSS

SEQ ID NO: 74 - protein, 133 aa, synthetic construct
  REGION 1..133: note = A3 heavy chain
EVQLVESGGGLVQPGGSLRLSCAASGFIFNRHWMHWVRQGPGKGLVWVSRINSDGSSTSYADSVKGRFTISRDNAKNTLHLQINSLRAEDTAVYYCARDGVRYYYDSTGYYPDSYYEYGMDVWGQGTTVTVSS

SEQ ID NO: 75 - protein, 133 aa, synthetic construct
  REGION 1..133: note = A10 heavy chain
QVQLVQSGGALVKPGGSLRLSCVASGFTFGSHWMHWVRQAPGKGLVWVSRVNSDGSSTNYADFVKGRFTTSRDNAENTLYLEMNSLTADDTAVYYCVRDGVRYYYDSSGYYPDSFFKYGMDVWGQGTTVTVSS

SEQ ID NO: 76 - protein, 126 aa, synthetic construct
  REGION 1..126: note = B4 heavy chain
QVQLQESGPGLVRPSETLSLTCTVSGLSVSTYYWSWIRQPPGKGLEWIAYVYSRGGTNYNPSLESRVTISVDTATNQFSLRLRSVTAADTAVYFCARATNYFDSSGYFFAPWFDPWGQGILVTVSS

SEQ ID NO: 77 - protein, 122 aa, synthetic construct
  REGION 1..122: note = B6 heavy chain
QVQLVQSGAEVKKPGSSVKVSCKASGGTRSSYAISWVRRAPGRGLEWMGVIIPFFGTANYAQIFQGRLTITADESTSIANMELTSLTPEDTAIYYCASGGGGYAGYNWFDPWGQGTLVTVSS

SEQ ID NO: 78 - protein, 133 aa, synthetic construct
  REGION 1..133: note = D6 heavy chain
EVQLVQSGGGLIQPGGSLKLSCAASGFSFRNHWMHWVRQAPGKGLVWVSRVNSDGYSTSYADSVKGRFTISRDNAKNTLYLQMNSLRPEDTAVYFCARDGVRFYSDSTGYYPDNYFPYGMDVWGQGTTVTVSS

SEQ ID NO: 79 - protein, 118 aa, synthetic construct
  REGION 1..118: note = B2 heavy chain
EVQLVESGGGLVQPGGSLRLSCKVSGFTFKAYWMHWVRQAPGKGLVWVSRINGLGSSRDYADSVRGRFTISRDDAENTVYLQMNSLTAEDTAMYYCARDVXFHDSSGYYRXGFXAPWG

SEQ ID NO: 80 - protein, 133 aa, synthetic construct
  REGION 1..133: note = C4 heavy chain
EVQLVESGGGLVQPGGSLRLSCAASGFAFSNHWMHWVRQAPGKGLVWVSRINSDGSSTTYADSVKGRFTISRDNAKNTLSLELNSLRAEDTAIYYCARDGVRFYYDSTGYYPDPYFQYGLDVWGQGTTVTVSS

SEQ ID NO: 81 - protein, 129 aa, synthetic construct
  REGION 1..129: note = C7 heavy chain
EVQLVESGGGLVQPGASLRVSCAASGFTFSTYNMNWVRQAPGKGLEWVSYISSRSSTIYYADSVQGRFTISRDNAKNSLYLQMNSLRAEDTAVYYCARDIGHYYDSSGYFHYSFGMDVWGQGTTVTVSS

SEQ ID NO: 82 - protein, 127 aa, synthetic construct
  REGION 1..127: note = D5 heavy chain
EVQLVESGGGLVQPGGSLRLSCAASGFIFRNYWMHWVRQAPGKGLVWVSRINGLGSTTTYADSVEGRFTITRDDAKNTIFLQMNSLRAEDTAVYYCARDVNFYDSSGYYREGWFDSWGPGTTVTVSS

SEQ ID NO: 83 - protein, 126 aa, synthetic construct
  REGION 1..126: note = D11 heavy chain
EVQLLESGAEVKKPGSSVKISCKASGGTFSNYAISWVRQAPGRGLEWLGGIIPIFGTPNYAQRFQGRVTITADESTSTAYMELNSLTSDDTAIYYCARDHPTVINPTFVGSWFDPWGQGTLVTVSS

SEQ ID NO: 84 - protein, 131 aa, synthetic construct
  REGION 1..131: note = B6 heavy chain
QVQLVESGAEVKKPGASVKVSCKASGFTFTSYYIHWVRQAPGQGLEWMGVINPSGGTTIYARNLQGRVTMTRDTSTTTVYMELSSLKSEDTAVYYCARAHSGNYDFWSGSNYHYYYGMDVWGQGTTVTVSS

SEQ ID NO: 85 - protein, 131 aa, synthetic construct
  REGION 1..131: note = D2 heavy chain
EVQLVESGAEVKKPGASVKVSCKASGFTFTSYYIHWVRQAPGQGLEWMGVINPSGGTTIYAQNFQGRVTMTRDTSTTTVYMELSSLKSEDTAVYYCARAHSGNYDFWSGSNYHYYYGMDVWGQGTTVTVSS

SEQ ID NO: 86 - protein, 109 aa, synthetic construct
  REGION 1..109: note = B3 light chain
QTVVTQEPSLTVSPGGTVTLTCGSNTGPVTNGHYPYWFQQKSGQAPRTLIYDTTNRQSWTPVRFSGSLLGGKAALTLSGAQPEDEADYHCLLSYSDGLVFGGGTKLTVL

SEQ ID NO: 87 - protein, 110 aa, synthetic construct
  REGION 1..110: note = A12 light chain
CMTPAPSTLAVTPGEPASISCRSTQSLLHSDGYNYLDWYLQKPGQSPHLLIYLGSHRASGVPDRFSGSGSDTDFTLKISRVEAEDVGVYYCMQPLRTPPTFGQGTKLEIK

SEQ ID NO: 88 - protein, 108 aa, synthetic construct
  REGION 1..108: note = B10 light chain
EIVLTQSPATLSLSAGDRATLSCRASQDISSFLAWYQQKPGQAPRLLMYDTSNRATGVPARFSGSRSGTDFTLTISTLEPEDVAVYYCQHRYNWPPYTFGQGTKVEIK

SEQ ID NO: 89 - protein, 108 aa, synthetic construct
  REGION 1..108: note = B11 light chain
EIVLTQSPATLSLSPGERATLSCRASQSISSFLAWYQQKPGQAPRLLIYDASNRVTGVPARFSGSRSGTDFTLTISTLEPEDFAVYYCQHRYNWPPYTFGQGTKVEIK

SEQ ID NO: 90 - protein, 108 aa, synthetic construct
  REGION 1..108: note = C9 light chain
EIVLTQSPATLSLSPGERATLSCRASQSISTYLAWYQQKPGQAPRLLIYDASNRATGVPARFSGSRSGTDFTLTISTLEPEDFAVYYCQQRYNWPPYTFGQGTKVEIK

SEQ ID NO: 91 - protein, 107 aa, synthetic construct
  REGION 1..107: note = A2 light chain
DIQMTQSPSSLSASVGDRVTITCRASQTISGSLSWYQHKPGKAPKLLIYAASSLQSGVPSRFSGSGSGTDFTLTISSLQPEDFATFYCQQSYSTPYTFGQGTKVEIK

SEQ ID NO: 92 - protein, 107 aa, synthetic construct
  REGION 1..107: note = A5 light chain
DIQMTQSPSSLSASIGDRVTITCRASESISSQLHWYQQKPGKAPRLLIYAASSLQGGVPSRFSGSGSGTDFTLTISGLQPEDFATYCCQQSFTTPYTFGQGTKVEIK

SEQ ID NO: 93 - protein, 108 aa, synthetic construct
  REGION 1..108: note = A7 light chain
EIVMTQSPATLSASPGERATLSCRASQDVSTFVAWFQQNPGQAPRLLIYDASTRAPGIPARFSGSRSGTEFTLTINSLQSEDFAVYYCQQYYNWPPWTFGQGTKVEIK

SEQ ID NO: 94 - protein, 107 aa, synthetic construct
  REGION 1..107: note = A8 light chain
DIQMTQSPSSVSASVGDRVTISCRASQDISASLGWYQQKPGKAPKLLIYRASNLEGGVPSRFRGSGSGTDFTLTISSLQPEDFATYYCLQANSFPLTFGGGTKVEIK

SEQ ID NO: 95 - protein, 107 aa, synthetic construct
  REGION 1..107: note = B10 light chain
DIQMTQSPSSLSASVGDSVTVACRASQPIYRNLNWYQQKPGKAPKLLIYDASTLQSGVPARFSGSGSGTDFTLTISSLQAEDFATYYCQQSYSSPRTFGQGTKVEIK

SEQ ID NO: 96 - protein, 109 aa, synthetic construct
  REGION 1..109: note = C2 light chain
DIQMTQSPSTLSASVGDRVTITCRASQSISTYLAWYQQKPGKAPKLLIYKASSLEIGVPSRFSGSGSGTEFTLTISSLQPDDFAIYYCQQYNNYSPPVTFGGGTKVEIK

SEQ ID NO: 97 - protein, 109 aa, synthetic construct
  REGION 1..109: note = D4 light chain
DIQMTQSPSTLSASVGDRVTITCRASQSISTYLAWYQQKPGKAPKLLIYKASTLESGVPLRFSGSGSGTEFTLTISSLQPDDFAIYYCQQYNNYSPPVTFGGGTKVEIK

SEQ ID NO: 98 - protein, 107 aa, synthetic construct
  REGION 1..107: note = B11 light chain
DIQMTQSPSSLSASVGDAVSITCRASESVSRQLNWYQQKPGKAPNLLIYAASSLQGGVPSRFSGSGSGTDFTLTISGLQPEDFATYYCQQGYSTPYSFGQGTKVEIK

SEQ ID NO: 99 - protein, 108 aa, synthetic construct
  REGION 1..108: note = A2 light chain
EIVLTQSPATLSLSAGERATLSCRASQSISSYLAWYQQKPGQAPRLLIYDASNRATGVPARFSGSQSGTDFTLTISTLEPEDFAVYYCQLRYNWPPYTFGQGTKVEIK

SEQ ID NO: 100 - protein, 107 aa, synthetic construct
  REGION 1..107: note = A4 light chain
DIQMTQSPSPLSASVGDRVTITCRASQSISSHLNWYQQKSGKVPKLLIYAASSLQSGVPSRFSGSGSGTDFTLTITSLQPEDFATYYCQQSDTTPYTFGQGTKVEIK

SEQ ID NO: 101 - protein, 107 aa, synthetic construct
  REGION 1..107: note = A5 light chain
DIQMTQSPSSLSASVGDAVSITCRASESIARQLNWYQQKPGKAPNLLIYAASSLQGGVPSRFSGSGSGADFTLTISGLQPEDFATYYCQQGYSTPYTFGQGTKVEIK

SEQ ID NO: 102 - protein, 108 aa, synthetic construct
  REGION 1..108: note = A9 light chain
EIVLTQSPATLSLSAGERATLSCRASQDISTFLAWYQQKPGQAPRLLIYDTSTRATGVPARFSGSRSGTDFTLTITTLEPEDFAVYYCQHRYNWPPYTFGQGTKVEIK

SEQ ID NO: 103 - protein, 108 aa, synthetic construct
  REGION 1..108: note = B2 light chain
EIVLTQSPATLSLSAGERATLSCRASQSISSYLAWYQQKPGQAPRLLIYDASNRATGVPARFSGSRSGTDFTLTISTLEPEDFAVYYCQHRYNWPPYTFGQGTKVEIK

SEQ ID NO: 104 - protein, 108 aa, synthetic construct
  REGION 1..108: note = B3 light chain
EIVLTQSPATLSLSPGERATLSCRASHSISTFLAWYQQKPGQAPRLLIYDTSTRATGVPARFSGSRSGTDFTLTINTLEPEDFAVYYCQQRYNWPPYTFGQGTKVEIK

SEQ ID NO: 105 - protein, 108 aa, synthetic construct
  REGION 1..108: note = B4 light chain
EIVLTQSPATLSLSPGERATLSCRASQSISSFLAWYQQKPGQAPRLLIYDTSNRATGVPARFSGSRSGTDFTLTISTLEPEDFAIYYCQHRYNWPPYTFGQGTKVEIK

SEQ ID NO: 106 - protein, 107 aa, synthetic construct
  REGION 1..107: note = B7 light chain
DIQMTQSPSSLSASVGDRVTITCRASQSISRSLNWYQQKPGKAPKLLIYAASTLQSGVPSRFSGSGSGTDFALTISSLQPEDFATYSCQQSDRTPYTFGQGTKVEIK

SEQ ID NO: 107 - protein, 108 aa, synthetic construct
  REGION 1..108: note = B11 light chain
EIVLTQSPATLSLSPGERATLSCRASQSISTYLVWYQQKPGQAPRLLIYDASTRATGVPARFSGSRSGTDFTLTISTLEPEDFAVYYCQHRYNWPPYTFGRGTKVEIK

SEQ ID NO: 108 - protein, 109 aa, synthetic construct
  REGION 1..109: note = C4 light chain
DIQMTQSPSTLSASVGDRVTITCRASQSISTYLAWYQQKVGKAPKLLIYKASTLEGGVPSRFSGSGSGTEFTLTISSLQPEDFAIYYCQQYNNYSPPVTFGGGTKVEIK

SEQ ID NO: 109 - protein, 112 aa, synthetic construct
  REGION 1..112: note = B10 light chain
DIVMTQSPLSLSVTPGEPASISCRSSQSLVYSDGNKYLDWYVQKPGQSPQLLIYLTSTRASGVPDRFSGSASGTDFTLKISRVEAEDVGLYYCMQALQTPFTFGPGTKVDIK

SEQ ID NO: 110 - protein, 108 aa, synthetic construct
  REGION 1..108: note = P6A1 ligth chain
EIVMTQSPATLSVSPGERATLTCRASQTISTFLAWYQQKPGQPPRLLIYDTSTRATGIPGRFSGSRSGTEFTLTISSLQSEDVAVYYCQHYYNWPPWTFGQGTKVEIK

SEQ ID NO: 111 - protein, 109 aa, synthetic construct
  REGION 1..109: note = P6A3 light chain
QSALTQPPSASGSPGQSVTISCTGSSSDIGGNEYVSWYQLQPGKAPKLMIYEVTKRPSGVPNRFSGSKSGNTASLTVSGLQSEDEGDYYCSSYADNSVLFGGGTTLTVL

SEQ ID NO: 112 - protein, 110 aa, synthetic construct
  REGION 1..110: note = P6A12 light chain
QSVLTQPPSASGSPGQSVTISCTGTSSDVGAYYYVSWYQQHPGKAPKLIIYEVNKRPSGVPARFSGSKSGNTASLTVSGLQGEDEADYYCTSYAGSNTVIFGGGTKLTVL

SEQ ID NO: 113 - protein, 108 aa, synthetic construct
  REGION 1..108: note = P6B4 light chain
EIVLTQSPVTLSLSPGERATLSCRASQTVDSTYLAWYQQKPGRAPRLLIYGASNRAIGVPSRFTGSGSGTDFTLTISRLEPEDFALYYCQQSDGSLFTFGPGTKVDIK

SEQ ID NO: 114 - protein, 107 aa, synthetic construct
  REGION 1..107: note = P6B5 light chain
DIQMTQSPASVSASVGDRVTISCRASQGIASWLAWYQQKPGKAPRLLIYGASSLQSGVPSRFRGSGSGTDFTLTISSLQPEDFATYYCQQANSFPFTFGPGTKVDIK

SEQ ID NO: 115 - protein, 110 aa, synthetic construct
  REGION 1..110: note = P6B11 light chain
QSALTQPASVSGSPGQSITISCTGTSSDVGRYNVVSWYQQHPGKAPKLIIYGSTKRPSGVSYRFSASKSGNTASLTISGLQAEDEAEYHCCSYASGSVWVFGGGTKLTVL

SEQ ID NO: 116 - protein, 110 aa, synthetic construct
  REGION 1..110: note = P6C4 light chain
QSALTQPPSASGSPGQSVTISCTGTSSDVGGYNYVSWYQHHPGKAPKLIIYEVSKRPSGVPHRFSGSKSGNTASLTVSGLQAEDEAEYYCSSYAGSNTFTFGGGTKLTVL

SEQ ID NO: 117 - protein, 110 aa, synthetic construct
  REGION 1..110: note = B8 light chain
QSALTQTASVSGSPGQSITISCTGTSSDAEIYNLVSWYQQHPGKAPKLIIYEGSKRPSGVSNRFSASKSAGAASLRISGLQPEDEADYYCCSYATSKTLVFGGGTKLTVV

SEQ ID NO: 118 - protein, 112 aa, synthetic construct
  REGION 1..112: note = C2 light chain
DVVMTQSPLSLPVTLGQPASISCRSSRSLLNSDGNTYLNWFHQRPGQSPRRLIFKLSNRDSGVPDRFSGSGSGTDFTLKISRVEAEDVGIYYCMQGTHWPVTFGGGTKVEIK

SEQ ID NO: 119 - protein, 110 aa, synthetic construct
  REGION 1..110: note = D8 light chain
QSALTQPASVSGSPGQSITISCTGTSSGVGSYNLVSWYQQHPGKAPKFIIYEGSKRPSGVSNRFSGSNSGNTASLTISGLQAEDEADYYCCSYAGSKTLVFGGGTKVTVL

SEQ ID NO: 120 - protein, 110 aa, synthetic construct
  REGION 1..110: note = A3 light chain
QSVLTQPASVSGSPGQSITISCTGTSSDVGSYNLVSWYQQHPGKAPKFIIYEGSKRPSGVSNRFSGSNSGNTASLTISGLQAEDEADYYCCSYAGSKTLVFGGGTKVTVL

SEQ ID NO: 121 - protein, 110 aa, synthetic construct
  REGION 1..110: note = A10 light chain
QSALTQPASVSGSPGQSITISCTGTSSDIGIYNLVSWYQQHPGKAPKLIIYEGSKRPSGVSNRFSASKSAGAASLTISGLQPEDEADYYCCSYATSKTLVFGGGTKLTVV

SEQ ID NO: 122 - protein, 107 aa, synthetic construct
  REGION 1..107: note = B4 light chain
EIVMTQSPATLSVSPGERATLSCRASQSVKSNLAWYQQKPGQAPRLLMYGASTRVVTIPARFSGSGSGTEFTLTISSLQSEDFAVYYCQQYNKWPLTFGGGTKVEIK

SEQ ID NO: 123 - protein, 110 aa, synthetic construct
  REGION 1..110: note = B6 light chain
QSALTQPASVSGSPGQSITISCTGTSSDIGGFNYVSWYQQHPGKAPKVMIFDVSNRPSGVSNRFSGSKSGNTASLTISGLQAEDEADYYCSSYTTRTTYVFGTGTKVTVL

SEQ ID NO: 124 - protein, 110 aa, synthetic construct
  REGION 1..110: note = D6 light chain
QSALTQPASVSGSPGQSITISCSGFSSDVGGDKVVSWYEQHPGKVPKLIIYEGSKRPSGVSNRFSGSKSGNTASLTISGLQAEDEADYYCCSYAGPKTLVFGGGTKVTVL

SEQ ID NO: 125 - protein, 102 aa, synthetic construct
  REGION 1..102: note = B2 light chain
NSPLSLSASVGDRVTITCRASRTIDNFLHWYQQKPGKAPNLLIYAASSLQSGVPSRFRGSGSGTDFTLTINSVQPEDFATYYCQQSYTIPPTFGGGTKVEIR

SEQ ID NO: 126 - protein, 110 aa, synthetic construct
  REGION 1..110: note = C4 light chain
QSALTQPASVSGSLGQSITISYTGTAIDVGSYNLVSWYQQHPGKVPKLMIYEGSKRPSGVSNRFFGSKSGNTASLTISGLQSEDEAEYYCCSYGGSRTLLFGGGTKLTVL

SEQ ID NO: 127 - protein, 112 aa, synthetic construct
  REGION 1..112: note = C7 light chain
DIVMTQSPLSLPVTLGEPASISCRSSRSLLHSNGYNYLDWYLQKPGQSPQLLIYLGSNRASGVPDRFSGSGSGTDFTLKISRVEAEDVGVYYCMQARQTPVTFGGGTKVEIK

SEQ ID NO: 128 - protein, 101 aa, synthetic construct
  REGION 1..101: note = D5 light chain
GPFTLSASVGDRVTITCRASRSINTFLNWYQQKTGSAPKLLIYGASTLQSGVPSRFSGSGSGTDFALTITSLQPDDFAAYYCQQSYTTPLTFGGGTRVEIK

SEQ ID NO: 129 - protein, 108 aa, synthetic construct
  REGION 1..108: note = D11 light chain
SYELTQPPSVSVAPGKTATITCGGDNIGSKTVHWYQQKPGQAPLLVIYYNGDRPPGIPERFSGSNSGNTATLTITRVEAGDEADYCCQIWDSRSSHPVFGGGTKLTVL

SEQ ID NO: 130 - protein, 112 aa, synthetic construct
  REGION 1..112: note = B6 light chain
DIVMTQSPLSLPVTPGEPASISCRSSQSLLHTNGYNFLDWYVQKPGQSPQLLIYLGSSRASGVPDRFSGSGSGTDFTLKISRVEAEDVGLYYCMQALHTPRTFGQGTKVEIK

SEQ ID NO: 131 - protein, 112 aa, synthetic construct
  REGION 1..112: note = D2 light chain
DIVMTQSPLSLPVTPGEPASISCRSSQSLLHTNGYNFLDWYVQKPGQSPQLLIYLGSSRASGVPDRFSGSGSGTDFTLKISRVEAEDVGLYYCMQALQTPRTFGQGTKVEIK

SEQ ID NO: 132 - protein, 561 aa, synthetic construct
  REGION 1..561: note = Envelope ectodomain protein sequence DENV1
FHLTTRGGEPHMIVSKQERGKSLLFKTSAGVNMCTLIAMDLGELCEDTMTYKCPRITEAEPDDVDCWCNATDTWVTYGTCSQTGEHRRDKRSVALAPHVGLGLETRTETWMSSEGAWKQIQKVETWALRHPGFTVIALFLAHAIGTSITQKGIIFILLMLVTPSMAMRCVGIGNRDFVEGLSGATWVDVVLEHGSCVTTMAKNKPTLDIELLKTEVTNPAVLRKLCIEAKISNTTTDSRCPTQGEATLVEEQDANFVCRRTVVDRGWGNGCGLFGKGSLLTCAKFKCVTKLEGKIVQYENLKYSVIVTVHTGDQHQVGNETTEHGTIATITPQAPTSEIQLTDYGTLTLDCSPRTGLDFNEVVLLTMKEKSWLVHKQWFLDLPLPWTSGASTSQETWNRQDLLVTFKTAHAKKQEVVVLGSQEGAMHTALTGATEIQTSGTTTIFAGHLKCRLKMDKLTLKGMSYVMCTGSFKLEKEVAETQHGTVLVQVKYEGTDAPCKIPFSTQDEKGVTQNGRLITANPIVTDKEKPINIETEPPFGESYIIVGAGEKALKLSWFKKG

SEQ ID NO: 133 - protein, 395 aa, synthetic construct
  REGION 1..395: note = Envelope ectodomain protein sequence DENV2
MRCIGISNRDFVEGVSGGSWVDIVLEHGSCVTTMAKNKPTLDFELIKTEAKQPATLRKYCIEAKLTNTTTESRCPTQGEPSLNEEQDKRFICKHSMVDRGWGNGCGLFGKGGIVTCAKFTCKKNMEGKIVQPENLEYTIVITPHSGEEHAVGNDTGKHGKEIKITPQSSTTEAELTGYGTVTMECSPRTGLDFNEMVLLQMEDKAWLVHRQWFLDLPLPWLPGADTQGSNWIQKETLVTFKNPHAKKQDVVVLGSQEGAMHTALTGATEIQMSSGNLLFTGHLKCRLRMDKLQLKGMSYSMCTGKFKIVKEIAETQHGTIVIRVQYEGDGSPCKIPFEITDLEKRHVLGRLITVNPIVTEKDSPVNIEAEPPFGDSYIIVGVEPGQLKLNWFKRG

SEQ ID NO: 134 - protein, 559 aa, synthetic construct
  REGION 1..559: note = Envelope ectodomain protein sequence DENV3
FHLTSRDGEPRMIVGKNERGKSLLFKTASGINMCTLIAMDLGEMCDDTVTYKCPHITEVEPEDIDCWCNLTSTWVTYGTCNQAGEHRRDKRSVALAPHVGMGLDTRTQTWMSAEGAWRQVEKVETWALRHPGFTILALFLAHYIGTSLTQKVVIFILLMLVTPSMTMRCVGVGNRDFVEGLSGATWVDVVLEHGGCVTTMAKNKPTLDIELQKTEATQLATLRKLCIEGKITNITTDSRCPTQGEAILPEEQDQNYVCKHTYVDRGWGNGCGLFGKGSLVTCAKFQCLESIEGKVVQHENLKYTVIITVHTGDQHQVGNETQGVTAEITSQASTAEAILPEYGTLGLECSPRTGLDFNEMILLTMKNKAWMVHRQWFFDLPLPWTSGATTKTPTWNRKELLVTFKNAHAKKQEVVVLGSQEGAMHTALTGATEIQTSGGTSIFAGHLKCRLKMDKLKLKGMSYAMCLNTFVLKKEVSETQHGTILIKVEYKGEDAPCKIPFSTEDGQGKAHNGRLITANPVVTKKEEPVNIEAEPPFGESNIVIGIGDKALKINWYRKG

SEQ ID NO: 135 - protein, 561 aa, synthetic construct
  REGION 1..561: note = Envelope ectodomain protein sequence DENV4
FSLSTRDGEPLMIVAKHERGRPLLFKTTEGINKCTLIAMDLGEMCEDTVTYKCPLLVNTEPEDIDCWCNLTSTWVMYGTCTQSGERRREKRSVALTPHSGMGLETRAETWMSSEGAWKHAQRVESWILRNPGFALLAGFMAYMIGQTGIQRTVFFVLMMLVAPSYGMRCVGVGNRDFVEGVSGGAWVDLVLEHGGCVTTMAQGKPTLDFELTKTTAKEVALLRTYCIEASISNITTATRCPTQGEPYLKEEQDQQYICRRDVVDRGWGNGCGLFGKGGVVTCAKFSCSGKITGNLVQIENLEYTVVVTVHNGDTHAVGNDTSNHGVTAMITPRSPSVEVKLPDYGELTLDCEPRSGIDFNEMILMKMKKKTWLVHKQWFLDLPLPWTAGADTSEVHWNYKERMVTFKVPHAKRQDVTVLGSQEGAMHSALAGATEVDSGDGNHMFAGHLKCKVRMEKLRIKGMSYTMCSGKFSIDKEMAETQHGTTVVKVKYEGAGAPCKVPIEIRDVNKEKVVGRIISSTPLAENTNSVTNIELEPPFGDSYIVIGVGNSALTLHWFRKG

SEQ ID NO: 136 - DNA, 1683 bp, synthetic construct
  misc_feature 1..1683: note = Envelope ectodomain nucleotide sequence DENV1
  source 1..1683: mol_type = other DNA
ttccatttgaccacacgagggggagagccacacatgatagttagtaagcaggaaagaggaaagtcactcttgttcaagacctctgcaggtgtcaatatgtgcactctcattgcgatggatttgggagagttatgtgaggacacaatgacttacaaatgcccccggatcactgaggcggaaccagatgacgttgactgctggtgcaatgccacagacacatgggtgacctatgggacgtgttctcaaaccggtgaacaccgacgagacaaacgttccgtggcactggccccacacgtgggacttggtctagaaacaagaaccgaaacatggatgtcctctgaaggcgcctggaaacaaatacaaaaagtggagacttgggctttgagacacccaggattcacggtgatagctctttttttagcacatgccataggaacatccatcactcagaaagggatcattttcattctgctgatgctggtaacaccatcaatggccatgcgatgcgtgggaataggcaacagagacttcgttgaaggactgtcaggagcaacgtgggtggacgtggtattggagcatggaagctgcgtcaccaccatggcaaaaaataaaccaacattggacattgaactcttgaagacggaggtcacgaaccctgccgtcttgcgcaaattgtgcattgaagctaaaatatcaaacaccaccaccgattcaagatgtccaacacaaggagaggctacactggtggaagaacaagacgcgaactttgtgtgtcgacgaacggttgtggacagaggctggggcaatggctgcggactatttggaaaaggaagcctactgacgtgtgctaagttcaagtgtgtgacaaaactggaaggaaagatagttcaatatgaaaacttaaaatattcagtgatagtcactgtccacacaggggaccagcaccaggtgggaaacgagactacagaacatggaacaattgcaaccataacacctcaagctcctacgtcggaaatacagttgacagactacggaacccttacactggactgctcacccagaacagggctggactttaatgaggtggtgctattgacaatgaaagaaaaatcatggcttgtccacaaacaatggtttctagacttaccactgccttggacttcgggggcttcaacatcccaagagacttggaacagacaagatttgctggtcacattcaagacagctcatgcaaagaagcaggaagtagtcgtactgggatcacaggaaggagcaatgcacactgcgttgaccggggcgacagaaatccagacgtcaggaacgacaacaatctttgcaggacacctgaaatgcagattaaaaatggataaactgactttaaaagggatgtcatatgtgatgtgcacaggctcatttaagctagagaaggaagtggctgagacccagcatggaactgtcctagtgcaggttaaatacgaaggaacagatgcgccatgcaagatccccttttcgacccaagatgagaaaggagtgacccagaatgggagattgataacagccaatcccatagttactgacaaagaaaaaccaatcaacattgagacagaaccaccttttggtgagagctacatcatagtaggggcaggtgaaaaagctttgaaactaagctggttcaagaaagga

SEQ ID NO: 137 - DNA, 1683 bp, synthetic construct
  misc_feature 1..1683: note = Envelope ectodomain nucleotide sequence DENV2
  source 1..1683: mol_type = other DNA
ttccatttaaccacacgtaacggagaaccacacatgatcgtcagtagacaagagaaagggaaaagtcttctgtttaaaacagaggatggtgtgaacatgtgtaccctcatggccatggaccttggtgaattgtgtgaagatacaatcacgtacaagtgtccttttctcaggcagaatgaaccagaagacatagattgttggtgcaactctacgtccacatgggtaacttatgggacgtgtaccaccacaggagaacacagaagagaaaaaagatcagtggcactcgttccacatgtgggaatgggactggagacacgaactgaaacatggatgtcatcagaaggggcctggaaacatgcccagagaattgaaacttggatcttgagacatccaggctttaccataatggcagcaatcctggcatacaccataggaacgacacatttccaaagagccctgattttcatcttactgacagctgtcgctccttcaatgacaatgcgttgcataggaatatcaaatagagactttgtagaaggggtttcaggaggaagctgggttgacatagtcttagaacatggaagctgtgtgacgacgatggcaaaaaacaaaccaacattggattttgaactgataaaaacagaagccaaacaacctgccactctaaggaagtactgtatagaggcaaagctgaccaacacaacaacagattctcgctgcccaacacaaggagaacccagcctaaatgaagagcaggacaaaaggttcgtctgcaaacactccatggtggacagaggatggggaaatggatgtggattatttggaaaaggaggcattgtgacctgtgctatgttcacatgcaaaaagaacatgaaaggaaaagtcgtgcaaccagaaaacttggaatacaccattgtgataacacctcactcaggggaagagcatgcagtcggaaatgacacaggaaaacatggcaaggaaatcaaaataacaccacagagttccatcacagaagcagagttgacaggctatggcactgtcacgatggagtgctctccgagaacgggcctcgacttcaatgagatggtgttgctgcaaatggaaaataaagcttggctggtgcacaggcaatggttcctagacctgccgttgccatggctgcccggagcggacacacaaggatcaaattggatacagaaagagacattggtgactttcaaaaatccccatgcgaagaaacaggatgttgttgttttgggatcccaagaaggggccatgcacacagcactcacaggggccacagaaatccagatgtcatcaggaaacttactgttcacaggacatctcaagtgcaggctgaggatggacaaactacagctcaaaggaatgtcatactctatgtgcacaggaaagtttaaagttgtgaaggaaatagcagaaacacaacatggaacaatagttatcagagtacaatatgaaggggacggttctccatgtaagatcccttttgagataatggatttggaaaaaagacatgttttaggtcgcctgattacagtcaacccaatcgtaacagaaaaagatagcccagtcaacatagaagcagaacctccattcggagacagctacatcatcataggagtagagccgggacaattgaagctcaactggtttaagaaagga

SEQ ID NO: 138 - DNA, 1678 bp, synthetic construct
  misc_feature 1..1678: note = Envelope ectodomain nucleotide sequence DENV3
  source 1..1678: mol_type = other DNA
ttccacttaacttcacgagatggagagccgcgcatgattgtggggaagaatgaaagaggaaaatccctactttttaagacagcctctggaatcaacatgtgcacactcatagccatggatttgggagagatgtgtgatgacacggtcacttacaaatgcccccacattaccgaagtggagcctgaagacattgactgttggtgcaaccttacatcgacatgggtgacttatggaacatgcaatcaagctggagagcatagacgcgataagagatcagtggcgttagctccccatgtcggcatgggactggacacacgcactcaaacctggatgtcggctgaaggagcttggagacaagtcgagaaggtagagacatgggcccttaggcacccagggtttaccatactagccctatttcttgcccattacataggcacttccttgacccagaaagtggttatttttatactattaatgctggttaccccatccatgacaatgagatgtgtgggagtaggaaacagagattttgtggaaggcctatcgggagctacgtgggttgacgtggtgctcgagcacggtgggtgtgtgactaccatggctaagaacaagcccacgctggacatagagcttcagaagactgaggccactcagctggcgaccctaaggaagctatgcattgagggaaaaattaccaacataacaaccgactcaagatgtcccacccaaggggaagcgattttacctgaggagcaggaccagaactacgtgtgtaagcatacatacgtggacagaggctggggaaacggttgtggtttgtttggcaagggaagcttggtgacatgcgcgaaatttcaatgtttagaatcaatagagggaaaagtggtgcaacatgagaacctcaaatacaccgtcatcatcacagtgcacacaggagaccaacaccaggtgggaaatgaaacgcagggagttacggctgagataacatcccaggcatcaaccgctgaagccattttacctgaatatggaaccctcgggctagaatgctcaccacggacaggtttggatttcaatgaaatgattttattgacaatgaagaacaaagcatggatggtacatagacaatggttctttgacttacccctaccatggacatcaggagctacaacaaaaacaccaacttggaacaggaaagagcttcttgtgacatttaaaaatgcacatgcaaaaaagcaagaagtagttgtccttggatcacaagagggagcaatgcatacagcactgacaggagctacagagatccaaacctcaggaggcacaagtatttttgcggggcacttaaaatgtagactcaagatggacaaattgaaactcaaggggatgagctatgcaatgtgcttgaatacctttgtgttgaagaaagaagtctccgaaacgcagcatgggacaatactcattaaggttgagtacaaaggggaagatgcaccctgcaagattcctttctccacggaggatggacaagggaaagctcacaatggcagactgatcacagccaatccagtggtgaccaagaaggaggagcctgtcaacattgaggctgaacctccttttggggaaagtaatatagtaattggaattggagacaaagccctgaaaatcaactggtacaggaagggaa

SEQ ID NO: 139 - DNA, 1683 bp, synthetic construct
  misc_feature 1..1683: note = Envelope ectodomain nucleotide sequence DENV4
  source 1..1683: mol_type = other DNA
ttttccctcagcacaagagatggcgaacccctcatgatagtggcaaaacatgaaagggggagacctctcttgtttaagacaacagaggggatcaacaaatgcactctcattgccatggacttgggtgaaatgtgtgaggacactgtcacgtataaatgccccctactggtcaataccgaacctgaagacattgattgctggtgcaacctcacgtctacctgggtcatgtatgggacatgcacccagagcggagaacggagacgagagaagcgctcagtagctttaacaccacattcaggaatgggattggaaacaagagctgagacatggatgtcatcggaaggggcttggaagcatgctcagagagtagagagctggatactcagaaacccaggattcgcgctcttggcaggatttatggcttatatgattgggcaaacaggaatccagcgaactgtcttctttgtcctaatgatgctggtcgccccatcctacggaatgcgatgcgtaggagtaggaaacagagactttgtggaaggagtctcaggtggagcatgggtcgacctggtgctagaacatggaggatgcgtcacaaccatggcccagggaaaaccaaccttggattttgaactgactaagacaacagccaaggaagtggctctgttaagaacctattgcattgaagcctcaatatcaaacataactacggcaacaagatgtccaacgcaaggagagccttatctgaaagaggaacaggaccaacagtacatttgccggagagatgtggtagacagagggtggggcaatggctgtggcttgtttggaaaaggaggagttgtgacatgtgcgaagttttcatgttcggggaagataacaggcaatttggtccaaattgagaaccttgaatacacagtggttgtaacagtccacaatggagacacccatgcagtaggaaatgacacatccaatcatggagttacagccatgataactcccaggtcaccatcggtggaagtcaaattgccggactatggagaactaacactcgattgtgaacccaggtctggaattgactttaatgagatgattctgatgaaaatgaaaaagaaaacatggctcgtgcataagcaatggtttttggatctgcctcttccatggacagcaggagcagacacatcagaggttcactggaattacaaagagagaatggtgacatttaaggttcctcatgccaagagacaggatgtgacagtgctgggatctcaggaaggagccatgcattctgccctcgctggagccacagaagtggactccggtgatggaaatcacatgtttgcaggacatcttaagtgcaaagtccgtatggagaaattgagaatcaagggaatgtcatacacgatgtgttcaggaaagttttcaattgacaaagagatggcagaaacacagcatgggacaacagtggtgaaagtcaagtatgaaggtgctggagctccgtgtaaagtccccatagagataagagatgtaaacaaggaaaaagtggttgggcgtatcatctcatccacccctttggctgagaataccaacagtgtaaccaacatagaattagaacccccctttggggacagctacatagtgataggtgttggaaacagcgcattaacactccattggttcaggaaaggg

SEQ ID NO: 140 - protein, 110 aa, synthetic construct
  REGION 1..110: note = A11 light chain
QSVLTQPVSVSGSPGQSITISCTGTSSNADTYNLVSWYQQRPGKAPKLMIYEGTKRPSGVSNRFSASKSATAASLTISGLQPEDEADYYCCSYATSRTLVFGGGTKLTVV

SEQ ID NO: 141 - protein, 218 aa, synthetic construct
  REGION 1..218: note = B7 light chain
RSQSALTQPASVSGSPGQSITISCTGISSDVETYNLVSWYEQHPGKAPKLIIYEASKRPSGVSNRFSGSKSGNTASLAISGLQAEDEADYYCCSYAGGKSLVFGGGTRLTVLGQPKAAPSVTLFPPSSEELQANKATLVCLISDFYPGAVTVAWKADSSPVKAGVETTTPSKQSNNKYAASSYLSLTPEQWKSHRSYSCQVTHEGSTVEKTVAPTECS

SEQ ID NO: 142 - protein, 131 aa, synthetic construct; identical to SEQ ID NO: 3
  REGION 1..131: note = Variable heavy chain of A11

SEQ ID NO: 143 - protein, 131 aa, synthetic construct
  REGION 1..131: note = Variable heavy chain of B7
EVQLVESGGGLVQPGGSLKLSCAASGFTFSSHWMHWVRQAPGKGLVWVSRTNSDGSSTSYADSVKGRFMISRDNSKNTVYLHMNGLRAEDTAVYFCARDGVRYYYDSTGYYPDNFFQYGLDVWGQGTTVTV

SEQ ID NO: 144 - protein, 120 aa, synthetic construct; identical to SEQ ID NO: 1
  REGION 1..120: note = Variable heavy chain of C8

SEQ ID NO: 145 - protein, 108 aa, synthetic construct; identical to SEQ ID NO: 37
  REGION 1..108: note = Variable light chain of C8

SEQ ID NO: 146 - protein, 126 aa, synthetic construct; identical to SEQ ID NO: 2
  REGION 1..126: note = Variable heavy chain of C10

SEQ ID NO: 147 - protein, 110 aa, synthetic construct; identical to SEQ ID NO: 38
  REGION 1..110: note = Variable light chain of C10

SEQ ID NO: 148 - protein, 12 aa, synthetic construct
  REGION 1..12: note = 150 loop of Denv-1
QHQVGNETTEHG

SEQ ID NO: 149 - protein, 12 aa, synthetic construct
  REGION 1..12: note = 150 loop of Denv-2
EHAVGNDTGKHG

SEQ ID NO: 150 - protein, 10 aa, synthetic construct
  REGION 1..10: note = 150 loop of Denv-3
QHQVGNETQG

SEQ ID NO: 151 - protein, 12 aa, synthetic construct
  REGION 1..12: note = 150 loop of Denv-4
THAVGNDIPNHG

SEQ ID NO: 152 - protein, 122 aa, synthetic construct
  REGION 1..122: note = C8 heavy chain
EVQLVESGGGLVQPGGSLRLSCSASGFTFSTYSMHWVRQAPGKGLEYVSAITGEGDSAFYADSVKGRFTISRDNSKNTLYFEMNSLRPEDTAVYYCVGGYSNFYYYYTMDVWGQGTTVTVSS

SEQ ID NO: 153 - protein, 128 aa, synthetic construct
  REGION 1..128: note = C10 heavy chain
EVQLVESGAEVKKPGASVKVSCKASGYTFTSYAMHWVRQAPGQRLEWMGWINAGNGNTKYSQKFQDRVTITRDTSASTAYMELSSLRSEDTAIYYCARDKVDDYGDYWFPTLWYFDYWGQGTLVTVSS

SEQ ID NO: 154 - protein, 133 aa, synthetic construct
  REGION 1..133: note = A11 heavy chain
EVQLVESGGGLVRPGGSLRLSCAASGFSYSNHWMHWVRQAPGKGLVWVSRINSDGSTRNYADFVKGRFTISRDNAENTLYLEMNSLTADDTAVYYCVRDGVRFYYDSTGYYPDSFFKYGMDVWGQGTTVTVSS

SEQ ID NO: 155 - protein, 133 aa, synthetic construct
  REGION 1..133: note = B7 heavy chain
EVQLVESGGGLVQPGGSLKLSCAASGFTFSSHWMHWVRQAPGKGLVWVSRTNSDGSSTSYADSVKGRFMISRDNSKNTVYLHMNGLRAEDTAVYFCARDGVRYYYDSTGYYPDNFFQYGLDVWGQGTTVTVSS

SEQ ID NO: 156 - protein, 129 aa, synthetic construct
  REGION 1..129: note = B7 light chain
QVQLQESGPGLMKPSETLSLTCSVSGVSISTHYWSWIRQPPGKGLEWIGFIYNSGGTHYNPSLKSRVTISADTSKNQFALTLSSVTAADTAVYYCARGRRAYDSSGYVKYYYFYGVDVWGQGTTVTVSS